European Patent Specification EP 3 684 914 B1, published May 29, 2024. Title: Tissue-specific expression of DELLA polypeptides. Applicant: Futuragene Israel Ltd. The sequence listing filed with the application follows.

SEQUENCE LISTING (85 sequences)

SEQ ID NO: 1 - protein, 628 aa, Eucalyptus grandis x urophylla
MKRDHRDACSGGYGGGGGGEASGASKGEPPSSSSTHSMPGSGKAKMVMWGEDDQDPSGGGGGGMDELLAVLGYKVRSSDMAEVAQKLEQLEMVMGSAQEDGISHLSYDAVHYNPSDLSSWVQSMLFELNPPPPPQQVADAVLAAAESSSTIAQHHRSHLGSRSQTQTRTLSQTSAPTQTQSQVIFNDDSEYDLRAIPGVAAFPQGDSDFESAARKKMKTLNGGSNSLSSSSSSSAAGAAPSESTRPVVLVDTQETGVRLVHTLMACAEAVQQENLKLADALVKHIGLLAASQNGAMRKVATYFAEALARRIYRIYPNDGSLDSSCNDILQMHFYETCPYLKFAHFTANQAILEAFATASRVHVIDFGLKQGMQWPALMQALALRPGGPPAFRLTGIGPPQPNNTDALQQVGWKLAQLADTIGVEFEFRGFVANSLADLEPAMLDIRPPEVETVAVNSVFELHPLLARPGAIDKVLSSIKAMRPKIVTMVEQEANHNGPGFVDRFTEALHYYSSLFDSLEGSGVAPPNQDLVMSEVYLGRQICNVVACEGPDRVERHETLVQWQARMGSAGFDPVHLGSNAFKQASMLLALFAGGEGYRVEENDGCLMLGWHTRPLIATSAWQLAAATQ

SEQ ID NO: 2 - DNA, 1887 bp, Eucalyptus grandis x urophylla
atgaagagggatcatcgagacgcttgcagtggcggctatggcggcggcggtggcggggaggcgagcggcgcctcgaagggcgagcccccgtcgtcctcctccacccactcaatgcccggctctggcaaggccaagatggtgatgtggggcgaggacgaccaagatccgagcggcggtggcgggggcggcatggacgagctcctcgcggtgctcgggtacaaggtgaggtcgtcggacatggccgaggtggcgcagaagctggagcagctcgagatggtgatgggctctgctcaggaggacggcatctcgcacctgtcctacgacgccgtccactacaacccttccgatctctcctcgtgggtccagagcatgctcttcgagctcaacccccctccgccgccgcagcaggtggccgacgcggtcctcgctgcggccgagtcgtcttccaccatcgcgcagcaccaccgttcgcatctcgggtctcggtctcagacgcagactcggactctgagtcagacttcggctcccactcagacgcagtcccaggtcatcttcaacgacgactccgagtacgacttgagggcgattcccggcgtcgccgctttcccacagggcgactcggacttcgagagcgccgcccggaagaagatgaagaccctgaacggcgggtcgaattcgttgtcgtcctcgtcctcttcgtcggccgccggagcggcgccctccgagtcgacccggccggtcgtcctggtggacacgcaggagactggggtgcggctcgtccacacgctcatggcctgcgccgaggcggtccagcaggagaacctgaagctggccgatgcgctcgtcaagcacattggcctgctcgccgcttcgcagaacggcgcgatgcgcaaggtagcgacctacttcgccgaggcgctcgcccgccggatttaccgaatctaccccaacgacggcagcctcgactcctcgtgcaacgacatcctccagatgcacttctacgagacctgcccgtacctcaaattcgcccacttcactgccaatcaggcgattcttgaagccttcgccaccgccagccgcgtccacgtcatcgatttcggcctcaagcagggtatgcagtggccggccctcatgcaggctctggccctgaggcccggcggtccgcccgccttccggctcaccgggattggcccgccgcagccgaacaacaccgacgccttgcagcaggtcggctggaagctggctcaattggccgacactatcggggtcgagttcgaattccggggtttcgtggcgaattcgctggctgatctcgagcccgccatgctggacatccgccctcccgaggtcgagacggtggccgtcaactcggtgtttgagctccaccccctgctcgcccgaccgggggcgattgacaaggttctctcatcgatcaaggccatgagacctaagatagtgacgatggtggaacaggaggcgaatcacaatggcccggggttcgtggaccggttcacggaagctttgcattactactccagcctgttcgattcgctggaagggtctggggtggctcccccgaaccaggatctggtcatgtccgaggtctacttgggtcggcagatttgcaatgttgtggcctgcgaggggccggatcgagtggagcggcacgagacgttggtgcagtggcaggcgcggatgggatcggctgggttcgacccggtccatctcgggtccaacgcgttcaagcaggcgagcatgctgctggccctgttcgcaggtggagaaggttaccgggtcgaggaaaacgatggttgtctcatgctcggttggcacacgaggcctctgatcgccacttcggcgtggcaactcgctgctgcaactcagtga

SEQ ID NO: 3 - protein, 634 aa, Eucalyptus grandis x urophylla
MKREHHHLYPQTDPSTSASAAAGKSKMWDEDGCGGGGDDELLAVLGYKVRSSDMAEVAQKLEQLEEVMFSAQEDGLSHLASETVHYNPSDLSSWLESMLSEFNPLPPPPGGFGGGPLSVPVAAAPPRPQPVGDPFLPRAESSSITTVDFGADQRMQSSCGRSSQMNEPRPEIGSSGIVFDEESSSDYDLKAIPGKAVFGRAQAQAQAQAQTRTRLASTSSSSTSSSAVTAKRFKSSPSDAAVGAAPESSRPVVLVDSQENGVRLVHALMACADAVQQDNLSIAEALVKQIGFLAISQAGAMRKVATFFAEALARRIYRVYPQNPPLDHSLTDALQMHFYETCPYLKFAHFTANQAILEAFEGKSRVHVIDFSMNQGLQWPALMQALALRPGGPPTFRLTGIGPPAPDNSDRLQEVGWKLAQLAETIHVEFEYRGFVANSLADLDASILELRPSDAEAVAVNSVFELHKLLARPGAIEKVLGVVRQVRPAIVTVVEQEANHNGPVFVDRFNESLHYYSTLFDSLEGCASTQDKAMSEVYLGKQICNVVACEGADRVERHETLAQWRARLGGAGFVPAHLGSNAFKQASMLLALFAGGDGYRVEENGGCLTLGWHTRPLIATSAWRLGGPSAGAAH

SEQ ID NO: 4 - DNA, 1905 bp, Eucalyptus grandis x urophylla
atgaagcgagagcaccaccacctctatccccagacggacccctccacctcggcctccgccgccgccgggaagtccaagatgtgggacgaagacggctgcggcggcggcggcgacgatgagctcctggccgtgctgggctacaaggtgcggtcctccgacatggccgaggttgcccagaagctggagcagctcgaggaggtcatgttcagcgcccaggaggacggcctctcccacctcgcctccgagaccgtccactacaacccctctgacctctcctcctggctcgagagcatgctgtccgagtttaatcccctgccgccgccccccggcgggttcggcggcggacccctctccgtccccgtcgccgccgcgccgccgcggccgcagcccgtgggcgacccgttcctcccccgcgcggagtcctcctccatcaccaccgttgacttcggggcggaccagcggatgcagagcagctgcgggaggagctcgcagatgaacgagccgcgcccggagatcggctcgtccgggatcgtgttcgatgaggagtcgtcttccgattacgatctcaaggctattcccggtaaggccgtgttcggccgcgcccaagcgcaagcgcaagcgcaagcgcagacccgcacccgcctcgcttctacgtcttcttcttccacctcctcgagcgccgtcaccgccaagcgcttcaaatcctctcccagcgacgcggccgtcggagccgccccggaatcgagccggccggtcgtcctggtggactcgcaggagaatggggtccggctcgtgcacgcgctcatggcctgcgcggatgccgtccagcaggacaacctcagcatcgcggaggcgctggtgaagcaaatcgggttcctggcgatctcgcaggccggggcgatgaggaaggtcgccactttcttcgcggaggcgctggcgcggcggatctaccgggtctacccgcagaacccgccgttggaccactccctcaccgacgccctccagatgcacttctacgagacctgtccttacctcaaattcgcccacttcaccgcgaaccaggccatcttggaggccttcgagggcaagagccgcgtccacgtcatcgacttcagcatgaaccagggcctccagtggccggcgctgatgcaggccctcgccctccgccccggtgggccgcccaccttccgcctcacggggatcggcccccccgccccggacaactccgaccgcctccaggaggtggggtggaagctggcccagctggcggagaccatccacgtcgagttcgagtaccgcgggttcgtcgccaacagcctcgccgacctcgacgcgtcgatcctggagctgcggccgagcgacgccgaggcggtggcggtcaactcggtgttcgagctgcacaagctgctggcccgcccgggggcgatcgagaaggttctgggcgtggtgcggcaggtgcggccggcgatcgtgacggtggtcgagcaggaggccaaccacaacgggccggtcttcgtggaccgcttcaacgagtcgctgcactactactccaccttgttcgactccctggagggctgcgccagcacgcaggacaaggccatgtcggaggtctacctcgggaagcagatctgcaacgtggtggcgtgcgagggcgccgaccgggtcgagcgccacgagaccctcgcccagtggcgggcccgcctcggcggcgccgggttcgtcccggcccacctcgggtcgaacgcgttcaagcaggcgagcatgctgctggccctgttcgccggcggggacgggtaccgggtggaggagaacggcggttgcctgacgctcgggtggcacacgcggccgctcatcgccacctcggcgtggcggctcggcggcccgagcgccggagccgcccactga

SEQ ID NO: 5 - protein, 567 aa, Eucalyptus grandis x urophylla
MGPFDPSAAAAAAAAAAVAASSSSSSSCSGGSAPKRHHHHHHHHPPPDLDGHLACAGYKVRSSELHHVAQRLERLETALVNSAAHIPHLASDAVHYNPSDLASWVDSMLSELPSSSFSSPCLPSGFPDPYSPAAAALGGGWVDQPSCSPHPQPHQNVVVPQQQQQQQQLTVVTALEEDSGIQLVHALMTCAESVQRGDASLAGSLVEEMRALLTRVDTSRGIGKVAGYFIDALGRRLLGLGSAPASAFENEVLYHHFYEACPYLKFAHFTANQAILEAFDGHDCVHVIDFNLMHGLQWPALIQALALRPRGPPLLRLTGIGPPSPDGRDALREIGLRLAELARSVNVRFAFRGVAASRLEDVKPWMLQVSPKEAVAVNSIMQLHRLLGSDPPRDPPIGSVLPWIRSLNPKIMTVAEQEANHNRPGFLDRFTEALYYYSTLFDSLEAACPVQPDKALAEMYLQREICNIVGCEGAARVERHEPLDRWRARLGRAGFRPLHLGSNAFKQASMLLTLFSTEGYSVEENEGCLTLCWHSRPLIAASAWQAAPTVVNSPAGVINHDDNNNQL

SEQ ID NO: 6 - DNA, 1704 bp, Eucalyptus grandis x urophylla
atgggccccttcgacccctccgccgccgccgccgccgccgccgcagcagccgtagccgccagcagctcctcgtcgtcgtcctgctccgggggctcggcgcccaagcgccaccaccaccaccaccaccaccacccgccgccggatctcgacgggcacctcgcctgcgccggctacaaggtccgctcctccgagctccaccacgtggcgcagcggctcgagcggctcgagaccgccctcgtcaactccgccgcccacatcccccacctcgcctccgacgctgtccactacaacccctccgatctcgcctcctgggtcgactccatgctctccgagctcccgagctcatccttctcctccccctgcctgccctccggcttccccgacccgtactctccggcggcggcggcactcggcggcgggtgggtggaccagccctcctgctcgccgcacccacagccgcaccagaacgtcgttgtcccccagcagcagcagcagcagcagcaattgacggtggtgacggcgctggaggaggattccggcattcagctcgtccacgcgctgatgacgtgtgcggagtcggtccagcgtggcgacgcctcgctggccggctccctggtcgaggagatgcgggccctgctgacgcgcgtcgacacctcgcggggcatcgggaaggtcgccggctacttcatcgacgccctcggccggcggctgctcggcctcggctcggctcccgcctccgccttcgagaacgaggtgctgtaccaccacttctacgaggcctgcccctatctcaagttcgcccacttcaccgccaaccaggccatcctcgaggccttcgacggccacgactgcgtccacgtcatcgacttcaacctcatgcacggcctgcagtggccggccctgatccaggccctcgccctccgcccccgcgggcccccgctcctccgcctcaccggcattggcccgccctcccccgacggccgcgacgctctccgcgagatcggcctccggctcgcggagctggcccgctcggtcaacgtccggttcgcgttccgcggcgtcgcggcctcgcggctcgaggacgtgaagccgtggatgctccaggtgagccccaaggaggccgtggccgtcaactccatcatgcagctccacaggctcctgggatccgacccgccccgggacccccccatcgggtcggtcctgccctggatccggagcctgaacccgaagataatgaccgtggcggagcaggaggcgaaccacaaccggcccgggttcctggaccggttcaccgaggcgctgtactactactcgaccctgttcgactcgctcgaggcggcctgcccggtccagcccgacaaggccctggccgagatgtaccttcaaagggagatatgcaacatcgtgggctgcgagggggcggcccgggtcgagaggcacgagccgctggaccggtggcgggcccgcctcgggcgagccgggttccggccgctgcacctcggctccaacgcgttcaagcaagccagcatgctgctcaccctgttctcgaccgagggctacagcgtggaggagaacgagggttgcttgacgctctgctggcacagccggcccctcatcgcggcttcggcgtggcaagccgcgcctactgtagtgaactcgccggccggcgttattaatcacgatgacaataataatcagctgtaa

SEQ ID NO: 7 - protein, 628 aa, Eucalyptus grandis
MKRDHRDACSGGYGGGGGGEASGASKGEPPSSSSTHSLPGSGKAKMVMWGEDDQDPSGGGGGGMDELLAVLGYKVRSSDMAEVAQKLEQLEMVMGSAQEDGISHLSYDAVHYNPSDLSSWVQSMLFELNPPPPPQQVADAVLAAAESSSTIAQHHRSHLGSRSQTQTRTLSQTSAPTQTQSQVIFNDDSEYDLRAIPGVAAFPQGDSDFESAARKKMKTLNGGSNSLSSSSSSSAAGAAPSESTRPVVLVDTQETGVRLVHTLMACAEAVQQENLKLADALVKHIGLLAASQNGAMRKVATYFAEALARRIYRIYPNDGSLDSSCNDILQMHFYETCPYLKFAHFTANQAILEAFATASRVHVIDFGLKQGMQWPALMQALALRPGGPPAFRLTGIGPPQPNNTDALQQVGWKLAQLADTIGVEFEFRGFVANSLADLEPAMLDIRPPEVETVAVNSVFELHPLLARPGAIDKVLSSIKAMRPKIVTMVEQEANHNGPGFVDRFTEALHYYSSLFDSLEGSGVAPPNQDLVMSEVYLGRQICNVVACEGPDRVERHETLVQWQARMGSAGFDPVHLGSNAFKQASMLLALFAGGEGYRVEENDGCLMLGWHTRPLIATSAWQLAAATQ

SEQ ID NO: 8 - DNA, 2147 bp, Eucalyptus grandis
atgaagagggatcatcgagacgcttgcagtggcggctatggcggcggcggtggcggggaggcgagcggcgcctcgaagggcgagcccccgtcgtcctcctccacccactcattgcccggctctggcaaggccaagatggtgatgtggggcgaggacgaccaagatccgagcggcggtggcgggggcggcatggacgagctcctcgcggtgctcgggtacaaggtgaggtcgtcggacatggccgaggtggcgcagaagctggagcagctcgagatggtgatgggctctgctcaggaggacggcatctcgcacctgtcctacgacgccgtccactacaacccttccgatctctcctcgtgggtccagagcatgctcttcgagctcaacccccctccgccgccgcagcaggtggccgacgcggtcctcgctgcggccgagtcgtcttccaccatcgcgcagcaccaccgttcgcatctcgggtctcggtctcagacgcagactcggactctgagtcagacttcggctcccactcagacgcagtcccaggtaatcttcaacgacgactccgagtacgacttgagggcgattcccggcgtcgccgctttcccacagggcgactcggacttcgagagcgccgcccggaagaagatgaagaccctgaacggcgggtcgaattcgttgtcgtcctcgtcctcttcgtcggccgccggagcggcgccctccgagtcgacccggccggtcgtcctggtggacacgcaggagactggggtgcggctcgtccacacgctcatggcctgcgccgaggcggtccagcaggagaacctgaagctggccgatgcgctcgtcaagcacattggcctgctcgccgcttcgcagaacggcgcgatgcgcaaggtagcgacctacttcgccgaggcgctcgcccgccggatttaccgaatctaccccaacgacggcagcctcgactcctcgtgcaacgacatcctccagatgcacttctacgagacctgcccgtacctcaaattcgcccacttcactgccaatcaggcgattcttgaagccttcgccaccgccagccgcgtccacgtcatcgatttcggcctcaagcagggtatgcagtggccggccctcatgcaggctctggccctgaggcccggcggtccgcccgccttccggctcaccgggattggcccgccgcagccgaacaacaccgacgccttgcagcaggtcggctggaagctggctcaattggccgacactatcggggtcgagttcgaattccggggtttcgtggcgaattcgctggctgatctcgagcccgccatgctggacatccgccctcccgaggtcgagacggtggccgtcaactcggtgtttgagctccaccccctgctcgcccgaccgggggcgattgacaaggttctctcatcgatcaaggccatgagacctaagatagtgacgatggtggaacaggaggcgaatcacaatggcccggggttcgtggaccggttcacggaagctttgcattactactccagcctgttcgattcgctggaagggtctggggtggctcccccgaaccaggatctggtcatgtccgaggtctacttgggtcggcagatttgcaatgttgtggcctgcgaggggccggatcgagtggagcggcacgagacgttggtgcagtggcaggcgcggatgggatcggctgggttcgacccggtccatctcgggtccaacgcgttcaagcaggcgagcatgctgctggccctgttcgcaggtggagaaggttaccgggtcgaggaaaacgatggttgtctcatgctcggttggcacacgaggcctctgatcgccacttcggcgtggcaactcgctgctgcaactcagtgaccgctggaccggtggcgggcccgcctcgggcgagccgggttccggccgctgcacctcggctccaacgcgttcaagcaagccagcatgctgctcaccctgttctcgaccgagggctacagcgtggaggagaacgagggttgcttgacgctctgctggcacagccggcccctcatcgcggcttcggcgtggcaagccgcgcctactgtagtgaactcgcggccggcgttattaatcacgatgacaataataatcagctgtaa

SEQ ID NO: 9 - protein, 628 aa, Eucalyptus grandis; identical to SEQ ID NO: 7

SEQ ID NO: 10 - DNA, 1904 bp, Eucalyptus grandis
atgaagcgagagcaccaccacctctatccccagacggacccctccacctcggcctccgccgccgccgggaagtccaagatgtgggacgaagacggctgcggcggcggcggcgacgatgagctcctggccgtgctgggctacaaggtgcggtcctccgacatggccgaggttgcccagaagctggagcagctcgaggaggtcatgttcagcgcccaggaggacggcctctcccacctcgcctccgagaccgtccactacaacccctctgacctctcctcctggctcgagagcatgctgtccgagtttaatcccctgccgccgccccccggcgggttcggcggcggacccctctccgtccccgtcgccgccgcgccgccgcggccgcagcccgtgggcgacccgttcctcccccgcgcggagtcctcctccatcaccaccgttgacttcggggcggaccagcggatgcagagcagctgcgggaggagctcgcagatgaacgagccgcccccggagatcggctcgtccgggatcgtgttcgatgaggagtcgtcttccgattacgatctcaaggctattcccggtaaggccgtgttcggccgcgcccaagcgcaagcgcaagcgcaagcgcagacccgcacccgcctcgcttctacgtcttcttcttccacctcctcgagcgccgtcaccgccaagcgcttcaaatcctctcccagcgacgcggccgtcggagccgccccggaatcgagccggccggtcgtcctggtggactcgcaggagaatggggtccggctcgtgcacgcgctcatggcctgcgcggatgccgtccagcaggacaacctcagcatcgcggaggcgctggtgaagcaaatcgggttcctggcgatctcgcaggccggggcgatgaggaaggtcgccactttcttcgcggaggcgctggcgcggcggatctaccgggtctacccgcagaacccgccgttggaccactccctcaccgacgccctccagatgcacttctacgagacctgtccttacctcaaattcgcccacttcaccgcgaaccaggccatcttggaggccttcgagggcaagagccgcgtccacgtcatcgacttcagcatgaaccagggcctccagtggccggcgctgatgcaggccctcgccctccgccccggtgggccgcccaccttccgcctcacggggatcggcccccccgccccggacaactccgaccgcctccaggaggtggggtggaagctggcccagctggcggagaccatccacgtcgagttcgagtaccgcgggttcgtcgccaacagcctcgccgacctcgacgcgtcgatcctggagctgcggccgagcgacgccgaggcggtggcggtcaactcggtgttcgagctgcacaagctgctggcccgcccgggggcgatcgagaaggttctgggcgtggtgcggcaggtgcggccggcgatcgtgacggtggtcgagcaggaggccaaccacaacgggccggtcttcgtggaccgcttcaacgagtcgctgcactactactccaccttgttcgactccctggagggctgcgccagcacgcaggacaaggccatgtcggaggtctacctcgggaagcagatctgcaacgtggtggcgtgcgagggcgccgaccgggtcgagcgccacgagaccctcgcccagtggcgggcccgcctcggcggcgccgggttcgtcccggcccacctcgggtcgaacgcgttcaagcaggcgagcatgctgctggccctgttcgccggcggggacgggtaccgggtggaggagaacggcggttgcctgacgctcgggtggcacacgcggccgctcatcgccactcggcgtggcggctcggcggcccgagcgccggagccgcccactga

SEQ ID NO: 11 - protein, 567 aa, Eucalyptus grandis
MGPFDPSAAAAAAAAAAASSSSSSSCSGGSAPKRHHHHHHHHPPPDLDGLLAGAGYKVRSSELHHVAQRLERLETALVNSAAHIPHLASDAVHYNPSDLASWVDSMLSELPSSSFSSPCLPSGFPDPYSPAAAALGGGWVDHPSCSPHPQPHQNVVVPQQPQPQQQQQLTVVTALEEDSGIQLVHALMTCAESVQRGDASLAGSLVEEMRALLTRVDTSRGIGKVAGYFIDALGRRLLGLGSAPASAFENEVLYHHFYEACPYLKFAHFTANQAILEAFDGHDCVHVIDFNLMHGLQWPALIQALALRPRGPPLLRLTGIGPPSPDGRDVLREIGLRLAELARSVNVRFAFRGVAASRLEDVKPWMLQVSPKEAVAVNSIMQLHRLLGSDPPRDPPIGSVLPWIRSLNPKIMTVAEQEANHNRPGFLDRFTEALYYYSTLFDSLEAACPVQPDKALAEMYLQREICNIVGCEGAARVERHEPLDRWRARLGRAGFRPLHLGSNAFKQASMLLTLFSTEGYSVEENEGCLTLCWHSRPLIAASAWQAAPTVVNSPAGVINHDDNNNQL

SEQ ID NO: 12 - DNA, 1704 bp, Eucalyptus grandis
atgggccccttcgacccctccgccgccgccgccgccgccgccgccgcagccgccagcagctcctcctcgtcgtcctgctccgggggctcggcgcccaagcgccaccaccaccaccaccaccaccacccgccgccggatctcgacgggctcctcgccggcgccggctacaaggtccgctcctccgagctccaccacgtggcgcagcggctcgagcggctcgagaccgccctcgtcaactccgccgcccacatcccccacctcgcctccgacgccgtccactacaacccctccgatctcgcctcctgggtcgactccatgctctccgagctcccgagctcatccttctcctccccctgcctgccctccggcttccccgacccgtactctccggcggcggcggcactcggcggcgggtgggtggaccacccctcctgctcgccgcacccacagccgcaccagaacgtcgtcgtcccccagcagccgcagccgcagcagcagcagcaattgacggtggtgacggcgctggaggaggattccggcattcagctcgtccacgcgctgatgacgtgcgcggagtcggtccagcgtggcgacgcctcgctggccggctccctggtcgaggagatgcgggccctgctgacgcgcgtcgacacctcgcggggcatcgggaaggtcgccggctacttcatcgacgccctcggccggcggctgctcggcctcggctcggctcccgcctcggccttcgagaacgaggtgctgtaccaccacttctacgaggcctgcccctatctcaagttcgcccacttcaccgccaaccaggccatcctcgaggccttcgacggccacgactgcgtccacgtcatcgacttcaacctcatgcacggcctgcagtggccggccctgatccaggccctcgccctccgcccccgcgggcccccgctcctccgcctcaccggcattggcccgccctcccccgacggccgcgacgtgctccgcgagatcggcctccggctcgcggagctggcccgctcggtcaacgtccggttcgcgttccgcggcgtcgcggcctcgcggctcgaggacgtgaagccgtggatgctccaggtgagccccaaggaggccgtggccgtcaactccatcatgcagctccacaggctcctgggatccgacccgccccgggacccccccatcgggtcggtcctgccctggatccggagcctgaacccgaagataatgaccgtggcggagcaggaggcgaaccacaaccggcccgggttcctggaccggttcaccgaggcgctgtactactactcgaccctgttcgactcgctcgaggcggcctgcccggtccagcccgacaaggccctggccgagatgtaccttcaaagggagatatgcaacatcgtgggctgcgagggggcggcccgggtcgagaggcacgagccgctggaccggtggcgggcccgcctcgggcgagccgggttccggccgctgcacctcggctccaacgcgttcaagcaagccagcatgctgctcaccctgttctcgaccgagggctacagcgtggaggagaacgagggttgcttgacgctctgctggcacagccggcccctcatcgcggcttcggcgtggcaagccgcgcctactgtagtgaactcgccggccggcgttattaatcacgatgacaataataatcagctgtaa

SEQ ID NO: 13 - protein, 533 aa, Arabidopsis thaliana
MKRDHHHHHHQDKKTMMMNEEDDGNGMDELLAVLGYKVRSSEMADVAQKLEQLEVMMSNVQEDDLSQLATETVHYNPAELYTWLDSMLTDLNPPSSNAEYDLKAIPGDAILNQFAIDSASSSNQGGGGDTYTTNKRLKCSNGVVETTTATAESTRHVVLVDSQENGVRLVHALLACAEAVQKENLTVAEALVKQIGFLAVSQIGAMRKVATYFAEALARRIYRLSPSQSPIDHSLSDTLQMHFYETCPYLKFAHFTANQAILEAFQGKKRVHVIDFSMSQGLQWPALMQALALRPGGPPVFRLTGIGPPAPDNFDYLHEVGCKLAHLAEAIHVEFEYRGFVANTLADLDASMLELRPSEIESVAVNSVFELHKLLGRPGAIDKVLGVVNQIKPEIFTVVEQESNHNSPIFLDRFTESLHYYSTLFDSLEGVPSGQDKVMSEVYLGKQICNVVACDGPDRVERHETLSQWRNRFGSAGFAAAHIGSNAFKQASMLLALFNGGEGYRVEESDGCLMLGWHTRPLIATSAWKLSTN

SEQ ID NO: 14 - DNA, 1602 bp, Arabidopsis thaliana
atgaagagagatcatcatcatcatcatcatcaagataagaagactatgatgatgaatgaagaagacgacggtaacggcatggatgagcttctagctgttcttggttacaaggttaggtcatccgaaatggctgatgttgctcagaaactcgagcagcttgaagttatgatgtctaatgttcaagaagacgatctttctcaactcgctactgagactgttcactataatccggcggagctttacacgtggcttgattctatgctcaccgaccttaatcctccgtcgtctaacgccgagtacgatcttaaagctattcccggtgacgcgattctcaatcagttcgctatcgattcggcttcttcgtctaaccaaggcggcggaggagatacgtatactacaaacaagcggttgaaatgctcaaacggcgtcgtggaaaccactacagcgacggctgagtcaactcggcatgttgtcctggttgactcgcaggagaacggtgtgcgtctcgttcacgcgcttttggcttgcgctgaagctgttcagaaagagaatctgactgtagcggaagctctggtgaagcaaatcggattcttagccgtttctcaaatcggagcgatgagaaaagtcgctacttacttcgccgaagctctcgcgcggcggatttaccgtctctctccgtcgcagagtccaatcgaccactctctctccgatactcttcagatgcacttctacgagacttgtccttatctcaagttcgctcacttcacggcgaatcaagcgattctcgaagcttttcaagggaagaaaagagttcatgtcattgatttctctatgagtcaaggtcttcaatggccggcgcttatgcaggctcttgcgcttcgacctggtggtcctcctgttttccggttaaccggaattggtccaccggcaccggataatttcgattatcttcatgaagttgggtgtaagctggctcatttagctgaggcgattcacgttgagtttgagtacagaggatttgtggctaacactttagctgatcttgatgcttcgatgcttgagcttagaccaagtgagattgaatctgttgcggttaactctgttttcgagcttcacaagctcttgggacgacctggtgcgatcgataaggttcttggtgtggtgaatcagattaaaccggagattttcactgtggttgagcaggaatcgaaccataatagtccgattttcttagatcggtttactgagtcgttgcattattactcgacgttgtttgactcgttggaaggtgtaccgagtggtcaagacaaggtcatgtcggaggtttacttgggtaaacagatctgcaacgttgtggcttgtgatggacctgaccgagttgagcgtcatgaaacgttgagtcagtggaggaaccggttcgggtctgctgggtttgcggctgcacatattggttcgaatgcgtttaagcaagcgagtatgcttttggctctgttcaacggcggtgagggttatcgggtggaggagagtgacggctgtctcatgttgggttggcacacacgaccgctcatagccacctcggcttggaaactctccaccaattag

SEQ ID NO: 15 - protein, 587 aa, Arabidopsis thaliana
MKRDHHQFQGRLSNHGTSSSSSSISKDKMMMVKKEEDGGGNMDDELLAVLGYKVRSSEMAEVALKLEQLETMMSNVQEDGLSHLATDTVHYNPSELYSWLDNMLSELNPPPLPASSNGLDPVLPSPEICGFPASDYDLKVIPGNAIYQFPAIDSSSSSNNQNKRLKSCSSPDSMVTSTSTGTQIGGVIGTTVTTTTTTTTAAGESTRSVILVDSQENGVRLVHALMACAEAIQQNNLTLAEALVKQIGCLAVSQAGAMRKVATYFAEALARRIYRLSPPQNQIDHCLSDTLQMHFYETCPYLKFAHFTANQAILEAFEGKKRVHVIDFSMNQGLQWPALMQALALREGGPPTFRLTGIGPPAPDNSDHLHEVGCKLAQLAEAIHVEFEYRGFVANSLADLDASMLELRPSDTEAVAVNSVFELHKLLGRPGGIEKVLGVVKQIKPVIFTVVEQESNHNGPVFLDRFTESLHYYSTLFDSLEGVPNSQDKVMSEVYLGKQICNLVACEGPDRVERHETLSQWGNRFGSSGLAPAHLGSNAFKQASMLLSVFNSGQGYRVEESNGCLMLGWHTRPLITTSAWKLSTAAY

SEQ ID NO: 16 - DNA, 1764 bp, Arabidopsis thaliana
atgaagagagatcatcaccaattccaaggtcgattgtccaaccacgggacttcttcttcatcatcatcaatctctaaagataagatgatgatggtgaaaaaagaagaagacggtggaggtaacatggacgacgagcttctcgctgttttaggttacaaagttaggtcatcggagatggcggaggttgctttgaaactcgaacaattagagacgatgatgagtaatgttcaagaagatggtttatctcatctcgcgacggatactgttcattataatccgtcggagctttattcttggcttgataatatgctctctgagcttaatcctcctcctcttccggcgagttctaacggtttagatccggttcttccttcgccggagatttgtggttttccggcttcggattatgaccttaaagtcattcccggaaacgcgatttatcagtttccggcgattgattcttcgtcttcgtcgaataatcagaacaagcgtttgaaatcatgctcgagtcctgattctatggttacatcgacttcgacgggtacgcagattggtggagtcataggaacgacggtgacgacaaccaccacgacaacgacggcggcgggtgagtcaactcgttctgttatcctggttgactcgcaagagaacggtgttcgtttagtccacgcgcttatggcttgtgcagaagcaatccagcagaacaatttgactctagcggaagctcttgtgaagcaaatcggatgcttagctgtgtctcaagccggagctatgagaaaagtggctacttacttcgccgaagctttagcgcggcggatctaccgtctctctccgccgcagaatcagatcgatcattgtctctccgatactcttcagatgcacttttacgagacttgtccttatcttaaattcgctcacttcacggcgaaccaagcgattctcgaagcttttgaaggtaagaagagagtacacgtcattgatttctcgatgaaccaaggtcttcaatggcctgcacttatgcaagctcttgcgcttcgagaaggaggtcctccaactttccggttaaccggaattggtccaccggcgccggataattctgatcatcttcatgaagttggttgtaaattagctcagcttgcggaggcgattcacgtagaattcgaataccgtggattcgttgctaacagcttagccgatctcgatgcttcgatgcttgagcttagaccgagcgatacggaagctgttgcggtgaactctgtttttgagctacataagctcttaggtcgtcccggtgggatagagaaagttctcggcgttgtgaaacagattaaaccggtgattttcacggtggttgagcaagaatcgaaccataacggaccggttttcttagaccggtttactgaatcgttacattattattcgactctgtttgattcgttggaaggagttccgaatagtcaagacaaagtcatgtctgaagtttacttagggaaacagatttgtaatctggtggcttgtgaaggtcctgacagagtcgagagacacgaaacgttgagtcaatggggaaaccggtttggttcgtccggtttagcgccggcacatcttgggtctaacgcgtttaagcaagcgagtatgcttttgtctgtgtttaatagtggccaaggttatcgtgtggaggagagtaatggatgtttgatgttgggttggcacactcgtccactcattaccacctccgcttggaaactctcgacggcggcgtactga

SEQ ID NO: 17 - protein, 511 aa, Arabidopsis thaliana
MKREHNHRESSAGEGGSSSMTTVIKEEAAGVDELLVVLGYKVRSSDMADVAHKLEQLEMVLGDGISNLSDETVHYNPSDLSGWVESMLSDLDPTRIQEKPDSEYDLRAIPGSAVYPRDEHVTRRSKRTRIESELSSTRSVVVLDSQETGVRLVHALLACAEAVQQNNLKLADALVKHVGLLASSQAGAMRKVATYFAEGLARRIYRIYPRDDVALSSFSDTLQIHFYESCPYLKFAHFTANQAILEVFATAEKVHVIDLGLNHGLQWPALIQALALRPNGPPDFRLTGIGYSLTDIQEVGWKLGQLASTIGVNFEFKSIALNNLSDLKPEMLDIRPGLESVAVNSVFELHRLLAHPGSIDKFLSTIKSIRPDIMTVVEQEANHNGTVFLDRFTESLHYYSSLFDSLEGPPSQDRVMSELFLGRQILNLVACEGEDRVERHETLNQWRNRFGLGGFKPVSIGSNAYKQASMLLALYAGADGYNVEENEGCLLLGWQTRPLIATSAWRINRVE

SEQ ID NO: 18 - DNA, 1536 bp, Arabidopsis thaliana
atgaagagagagcacaaccaccgtgaatcatccgccggagaaggtgggagttcatcaatgacgacggtgattaaagaagaagctgccggagttgacgagcttttggttgttttaggttacaaagttcgatcatccgacatggctgacgtggcacacaagcttgaacagttagagatggttcttggtgatggaatctcgaatctttctgatgaaactgttcattacaatccttctgatctctctggttgggtcgaaagcatgctctcggatcttgacccgacccggattcaagaaaagcctgactcagagtacgatcttagagctattcctggctctgcagtgtatccacgtgacgagcacgtgactcgtcggagcaagaggacgagaattgaatcggagttatcctctacgcgctctgtggtggttttggattctcaagaaactggagtgcgtttagtccacgcgctattagcttgtgctgaagctgttcaacagaacaatttgaagttagccgacgcgctcgtgaagcacgtggggttactcgcgtcctctcaagctggtgctatgaggaaagtcgcgacttacttcgctgaagggcttgcgagaaggatttaccgtatttaccctcgagacgatgtcgcgttgtcttcgttttcggacactcttcagattcatttctatgagtcttgtccgtatctcaagtttgcgcattttacggcgaatcaagcgatacttgaggtttttgctacggcggagaaggttcatgttattgatttaggacttaaccatggtttacaatggccggctttgattcaagctcttgctttacgtcctaatggtccaccggattttcggttaaccgggatcggttattcgttaaccgatattcaagaagttggttggaaacttggtcagcttgcgagtactattggtgtcaatttcgaattcaagagcattgctttaaacaatttgtctgatcttaaaccggaaatgctagacattagacccggtttagaatcagtggcggttaactcggtcttcgagcttcatcgcctcttagctcatcccggttccatcgataagtttttatcgacaatcaaatcaatccgaccggatataatgactgtggtcgagcaagaagcaaaccataacggtaccgtatttctcgatcggttcacggaatcgctacattactattcgagcttattcgactcgctcgagggcccgccaagccaagaccgagtgatgtcggagttattcctaggacggcagatactaaaccttgtggcatgcgaaggagaagaccgggtagagaggcatgagactttaaatcagtggagaaaccggttcggtttaggaggatttaaaccggttagtatcggttcgaacgcgtataagcaagcaagcatgttgttggcactttatgccggggctgatgggtataatgtggaagagaatgaaggttgtttgttgcttggatggcaaacgcgaccgcttattgcaacatctgcgtggcgaatcaatcgtgtggaataa

SEQ ID NO: 19 - protein, 547 aa, Arabidopsis thaliana
MKRGYGETWDPPPKPLPASRSGEGPSMADKKKADDDNNNSNMDDELLAVLGYKVRSSEMAEVAQKLEQLEMVLSNDDVGSTVLNDSVHYNPSDLSNWVESMLSELNNPASSDLDTTRSCVDRSEYDLRAIPGLSAFPKEEEVFDEEASSKRIRLGSWCESSDESTRSVVLVDSQETGVRLVHALVACAEAIHQENLNLADALVKRVGTLAGSQAGAMGKVATYFAQALARRIYRDYTAETDVCAAVNPSFEEVLEMHFYESCPYLKFAHFTANQAILEAVTTARRVHVIDLGLNQGMQWPALMQALALRPGGPPSFRLTGIGPPQTENSDSLQQLGWKLAQFAQNMGVEFEFKGLAAESLSDLEPEMFETRPESETLVVNSVFELHRLLARSGSIEKLLNTVKAIKPSIVTVVEQEANHNGIVFLDRFNEALHYYSSLFDSLEDSYSLPSQDRVMSEVYLGRQILNVVAAEGSDRVERHETAAQWRIRMKSAGFDPIHLGSSAFKQASMLLSLYATGDGYRVEENDGCLMIGWQTRPLITTSAWKLA

SEQ ID NO: 20 - DNA, 1644 bp, Arabidopsis thaliana
atgaagagaggatacggagaaacatgggatccgccaccaaaaccactaccagcttctcgttccggagaaggtccttcaatggcggataagaagaaggctgatgatgacaacaacaacagcaacatggatgatgagcttcttgctgttcttggctacaaggttcgatcttctgagatggctgaagtagcacagaagcttgaacaacttgagatggtcttgtctaatgatgatgttggttctactgtcttaaacgactctgttcattataacccatctgatctctctaactgggtcgagagcatgctttctgagctgaacaacccggcttcttcggatcttgacacgacccgaagttgtgtggatagatccgaatacgatctcagagcaattccgggtctttctgcgtttccaaaggaagaggaagtctttgacgaggaagctagcagcaagaggatccgactcggatcgtggtgcgaatcgtcggacgagtcaactcggtccgtggtgctcgttgactctcaggagaccggagttagacttgtccacgcactagtggcgtgcgctgaggcgattcaccaggagaatctcaacttagctgacgcgctggtgaaacgcgtgggaacactcgcgggttctcaagctggagctatgggaaaagtcgctacgtattttgctcaagccttggctcgtcgtatttaccgtgattacacggcggagacggacgtttgcgcggcggtgaacccatctttcgaagaggttttggagatgcacttttacgagtcttgcccttacctgaagttcgctcatttcacggcgaaccaagcgattctagaagctgttacgacggcgcgtagagttcacgtcattgatttagggcttaatcaagggatgcaatggcctgctttaatgcaagctttagctctccgacccggtggacctccgtcgtttcgtctcaccggaatcggaccaccgcagacggagaattcagattcgcttcaacagttaggttggaaattagctcaattcgctcagaacatgggcgttgaattcgaattcaaaggcttagccgctgagagtttatcggatcttgaacccgaaatgttcgaaacccgacccgaatctgaaaccttagtggttaattcggtatttgagctccaccggttattagcccgatccggttcaatcgaaaagcttctcaatacggttaaagctattaaaccgagtatcgtaacggtggttgagcaagaagcgaaccacaacggaatcgtcttcctcgataggttcaacgaagcgcttcattactactcgagcttgtttgactcgctcgaagacagttatagtttaccgagtcaagaccgagttatgtcagaagtgtacttagggagacagatactcaacgttgttgcggcggaagggtccgatcgggtcgagcggcacgagacggctgcacagtggaggattcggatgaaatccgctgggtttgacccgattcatctcggatctagcgcgtttaaacaagcgagtatgcttttatcgctttacgctaccggagatggatacagagttgaagaaaatgacggatgtttaatgatagggtggcagacgcgaccactcatcacaacctcggcgtggaaactcgcctga

SEQ ID NO: 21 - protein, 523 aa, Arabidopsis thaliana
MKRSHQETSVEEEAPSMVEKLENGCGGGGDDNMDEFLAVLGYKVRSSDMADVAQKLEQLEMVLSNDIASSSNAFNDTVHYNPSDLSGWAQSMLSDLNYYPDLDPNRICDLRPITDDDECCSSNSNSNKRIRLGPWCDSVTSESTRSVVLIEETGVRLVQALVACAEAVQLENLSLADALVKRVGLLAASQAGAMGKVATYFAEALARRIYRIHPSAAAIDPSFEEILQMNFYDSCPYLKFAHFTANQAILEAVTTSRVVHVIDLGLNQGMQWPALMQALALRPGGPPSFRLTGVGNPSNREGIQELGWKLAQLAQAIGVEFKFNGLTTERLSDLEPDMFETRTESETLVVNSVFELHPVLSQPGSIEKLLATVKAVKPGLVTVVEQEANHNGDVFLDRFNEALHYYSSLFDSLEDGVVIPSQDRVMSEVYLGRQILNLVATEGSDRIERHETLAQWRKRMGSAGFDPVNLGSDAFKQASLLLALSGGGDGYRVEENDGSLMLAWQTKPLIAASAWKLAAELRR

SEQ ID NO: 22 - DNA, 1572 bp, Arabidopsis thaliana
atgaaacgaagccatcaagaaacgtctgtagaagaagaagctccttcaatggtggagaagttagaaaatggttgtggtggtggtggagacgataacatggacgagtttcttgctgttttgggttacaaggttcgatcttcagacatggcagatgttgcacagaagcttgaacagcttgaaatggtcttgtccaatgatattgcctcttctagtaatgccttcaatgacaccgttcattacaatccttctgatctctccggttgggctcagagcatgctctcggatcttaattactacccggatcttgacccgaaccggatttgcgatctgagaccaatcacagacgacgatgagtgttgcagtagcaatagtaacagcaacaagaggattcgactcggtccttggtgtgactcagtgaccagcgagtcaactcgttccgtggtgcttatcgaggagacaggagttagactcgttcaggcgctagtggcctgcgccgaggcggttcagctggagaatctgagcctcgcggatgctctcgtcaagcgcgtgggattactcgcggcttctcaagccggagccatggggaaagtcgctacctacttcgccgaagccctagctcgtcgaatttaccggattcatccttccgccgccgccattgatccttccttcgaagagattcttcagatgaacttctacgactcgtgtccctacctgaaattcgctcatttcacggccaatcaggcgattctagaagctgttacgacgtcgcgtgtcgtacacgtaatcgatctagggcttaatcaaggtatgcaatggccggcgttaatgcaagccttagctctccgacccggtggtccaccgtcgtttcgtctcaccggcgttgggaatccgtcgaatcgagaagggattcaagagttaggttggaagctagctcagctggctcaagccatcggcgtcgaattcaaattcaatggtctaacgacggagaggttatccgatttagaaccggatatgttcgagacccgaaccgaatcggagactctagtggttaattcggttttcgagcttcacccggttttatcccaacccggttcgatcgaaaagctgttagcgacggttaaggcggttaaaccgggtctcgtaacagtggtggaacaagaagcgaaccataacggtgacgttttcttagaccggtttaacgaagcgcttcactattactcgagcttgttcgactcgctcgaagatggtgttgtgataccgagtcaagaccgagtcatgtcggaggtttacttagggagacagatattgaacttggtggcgacggaaggaagcgataggatcgagcgacacgagacgctggctcagtggcgaaaacgtatgggatccgccgggtttgacccggttaacctcggatcagacgcgtttaagcaagcgagtttgctattggcgttatctggcggtggagatggatacagagtggaggagaacgacggaagcctaatgcttgcgtggcaaacgaaacctctaatcgctgcatcggcgtggaaactagcggcggagttgcggcggtag

SEQ ID NO: 23 - DNA, 300 bp, Artificial Sequence
  Reverse complementary sequence of the DELLA1 300 bp sequences
agattgtgacgatggtggaacaggaggcgaatcacaatggcccggggttcgtggaccggttcacggaagctttgcattactactccagcctgttcgattcgctggaagggtctggggtggctcccccgaaccaggatctggtcatgtccgaggtctacttgggtcggcagatttgcaatgttgtggcctgcgaggggccggatcgagtggagcggcacgagacgttggtgcagtggcaggcgcggatgggatcggctgggttcgacccggtccatctcgggtccaacgcgttcaagcagg

SEQ ID NO: 24 - DNA, 396 bp, Artificial Sequence
  Reverse complementary sequence of the DELLA2 396 bp sequence
cagctcgaggaggtcatgttcagcgcccaggaggacggcctctcccacctcgcctccgagaccgtccactacaacccctctgacctctcctcctggctcgagagcatgctgtccgagtttaatcccctgccgccgccccccggcgggttcggcggcggacccctctccgtccccgtcgccgccgcgccgccgcggccgcagcccgtgggcgacccgttcctcccccgcgcggagtcctcctccatcaccaccgttgacttcggggcggaccagcggatgcagagcagctgcgggaggagctcgcagatgaacgagccgcgcccggagatcggctcgtccgggatcgtgttcgatgaggagtcgtcttccgattacgatctcaaggctattcccggt

SEQ ID NO: 25 - DNA, 300 bp, Artificial Sequence
  Reverse complementary sequence of the DELLA3 300 bp sequence
aggtgagccccaaggaggccgtggccgtcaactccatcatgcagctccacaggctcctgggatccgacccgccccgggacccccccatcgggtcggtcctgccctggatccggagcctgaacccgaagataatgaccgtggcggagcaggaggcgaaccacaaccggcccgggttcctggaccggttcaccgaggcgctgtactactactcgaccctgttcgactcgcttgaggcggcctgcccggtccagcccgacaaggccctggccgagatgtaccttcaaagggagatatgcaaca

SEQ ID NO: 26 - DNA, 108 bp, Artificial Sequence
  Partial random intron sequence
ggctcgaacgagccgactaattgtctttaaacgcgcgatataagcgcacaatgggcgcgccaaacgataaactctatcgctctgtcgcgtgcgtggcatcttcgcgcg

SEQ ID NO: 27 - DNA, 18 bp, Artificial Sequence
  Forward primer
gtgacgatggtggaacag

SEQ ID NO: 28 - DNA, 18 bp, Artificial Sequence
  Reverse primer
catgctcgcctgcttgaa

SEQ ID NO: 29 - DNA, 18 bp, Artificial Sequence
  Forward primer
ccccggacaactccgacc

SEQ ID NO: 30 - DNA, 16 bp, Artificial Sequence
  Reverse primer
cggtccacgaagaccg

SEQ ID NO: 31 - DNA, 21 bp, Artificial Sequence
  Forward primer
cctgaacccgaagataatgac

SEQ ID NO: 32 - DNA, 19 bp, Artificial Sequence
  Reverse primer
atgctggcttgcttgaacg

SEQ ID NO: 33 - DNA, 23 bp, Artificial Sequence
  Forward primer
cgaacgagccgactaattgtctt

SEQ ID NO: 34 - DNA, 18 bp, Artificial Sequence
  Reverse primer
cgcgcgaagatgccacgc

SEQ ID NO: 35 - DNA, 20 bp, Artificial Sequence
  Forward primer
agcttagccgatctcgatgc

SEQ ID NO: 36 - DNA, 20 bp, Artificial Sequence
  Reverse primer
tccacacgataaccttggcc

SEQ ID NO: 37 - DNA, 20 bp, Artificial Sequence
  Forward primer
agaaggtccttcaatggcgg

SEQ ID NO: 38 - DNA, 20 bp, Artificial Sequence
  Reverse primer
aacgcagaaagacccggaat

SEQ ID NO: 39 - DNA, 20 bp, Artificial Sequence
  Forward primer
gtgcaacgacatcctccaga

SEQ ID NO: 40 - DNA, 20 bp, Artificial Sequence
  Reverse primer
gcgaaggcttcaagaatcgc

SEQ ID NO: 41 - DNA, 914 bp, Artificial Sequence
  Constitutive promoter
agattagccttttcaatttcagaaagaatgctaacccacagatggttagagaggcttacgcagcaggtctcatcaagacgatctacccgagcaataatctccaggaaatcaaataccttcccaagaaggttaaagatgcagtcaaaagattcaggactaactgcatcaagaacacagagaaagatatatttctcaagatcagaagtactattccagtatggacgattcaaggcttgcttcacaaaccaaggcaagtaatagagattggagtctctaaaaaggtagttcccactgaatcaaaggccatggagtcaaagattcaaatagaggacctaacagaactcgccgtaaagactggcgaacagttcatacagagtctcttacgactcaatgacaagaagaaaatcttcgtcaacatggtggagcacgacacacttgtctactccaaaaatatcaaagatacagtctcagaagaccaaagggcaattgagacttttcaacaaagggtaatatccggaaacctcctcggattccattgcccagctatctgtcactttattgtgaagatagtggaaaaggaaggtggctcctacaaatgccatcattgcgataaaggaaaggccatcgttgaagatgcctctgccgacagtggtcccaaagatggacccccacccacgaggagcatcgtggaaaaagaagacgttccaaccacgtcttcaaagcaagtggattgatgtgatatctccactgacgtaagggatgacgcacaatcccactatccttcgcaagacccttcctctatataaggaagttcatttcatttggagagaacacgggggactctagatatttttacaacaattaccaacaacaacaaacaacaaacaacattacaattactatttacaattaca

SEQ ID NO: 42 - DNA, 301 bp, Artificial Sequence
  Constitutive promoter
tttacagtaagaactgataacaaaaattttacttatttccttagaattaatcttaaaggtgatagtaaacaaggacgattagtccgttggcaaaattggttcagcaagtatcaatttgatgtcgaacatcttgaaggtgtaaaaaacgttttagcagattgcctcacgagagattttaatgcttaaaaacgtaagcgctgacgtatgatttcaaaaaacgcagctataaaagaagccctccagcttcaaagttttcatcaacacaaattctaaaaacaaaattttttagagagggggagtg

SEQ ID NO: 43 - DNA, 1501 bp, Artificial Sequence
  Green tissue promoter
tgcgttatactaaagatattcagatcaatctatgtcaatctattcacgaaaacccggagagtctaatgaggagagttgcatcttggcaatatagtttttaagaatggatatccagatccctacgaactggattcacacagtcactgctgtaagctctggttttttttagcttaggaagcaggttatgatcaaacatgattaaaccatcgcgtgtttgccagccatcagaaatggaaaggcgaatgttgttatagtgatggacagatcatgctgagatgattgattatgaatcttactgatgactgtcatttatgttatcgcactctgtgtgcgtgggtgtgtgttatgagtaatatcaaattaaccagacgataggtgttgaagattagctgttgggccaccgtggcgaaaggtgtcttatacaagccatcggcagtgacgcagaactgtagagaaccgctctaacaagtcttcgaatgcattcttttaatgtacagcacgacatgaagggggttcgagtgtagcgaacagttcgtgcgagaaagatcattttcaatagcataaaagagtctgctttctgctgcaaacatggaaagaacttacatttcaatcattgaggagaagattataacaaatcctaaatggttgagattttagttagtccattcgaactaaagtggcgaagatgtcagtttttcaagtggatgatatttctcatgtatgttccgcagaggcaatcaccttgtttgtaactagacatctagagaacctaacaaggattgatgggggtgaggtgaaatgtctgtttcctctttaatatggatccagcgatgccttacagagcggatggatggcactggcaagtcttaatccttagctcgaatgtttgattggtaacagatgccttttctttcttttcaatcacagctgacaaatgcaaatatctaaaaccattggttgtttggtgcttgcaagtctggattaccccactttatgtttcacctttcaataatgaataacaaggtactcgggaaaaaaaggaaagggaaattcgcacaaccaaagttgctatgcagaagtcaactcaatcctaatcaagttgatgagagtgttgggccctattttctgcagcaaacatgaatctcgattcatctccctcgcaaaagataaggaagctgcaaaagctttcctcctaagtttgttggcaagcaaattgattttgtaccagaaataaatacaaagtgaaacccaagcaatcacgcatggcctgatttgtgccatgtccatttgatctccctctactatttttcctgctttctcaagcaaactagttgctgtaacagtgaatgatcccccggctctctctctctctctctctctctccatttattccatccatgtttttgcttttcgcacaacacttatcattgaggtgctaactactgaattcccctaactaaaaattggaacctctcacctaatttcattttctcccactttg

SEQ ID NO: 44 - DNA, 1149 bp, Artificial Sequence
  Root promoter
gccggctgatcatgtttattcttcgctaatgaaaaatatttagctctcaagggaccgtcaattcaggatcgtgaagttacgtgcgctagtaaagttcatcgactagtagtagatgcggatgacaagtaaatctacacaagcgagacataggcaagtcgtttcaacctcctatcccattcataattaatgaaatgagatcttctaaaacgagtcatcgcagtctgttcttctatctactaaccatatgatgtttgctttaataggcaagtcattccctcactctgcatgactttcataaatttttcaccgtctctgtgttacatttctttatcatagagcattaagactagatactgagataggcaaactagataccttcattatgcccccgaagatgaagccgagataaagaaattaacttgacatgaatcgggatggcaaacctctaagaacagtgggggcaaggttgggcaactcgcccggcccgctctacttcattccattccattccattccattaccattccattaccattaccattaccattcccattccccatatcttcatgaaaggttggtggacaatagtggtgcttatctcgatcgtacctttccgctattttattcatgcaaatagcccttcggcgcgtccattctcatgtcacgaggaaaatgacataaggacatgattagggtcgatggtcctttgcttccgcgaattattccctctaaaaccgcatttaataatctcccggaagagcgacagggactcgcttgtctcgttgcacgtaaattactagttaagctggttgtccttatgcccataatcgcccattattacacatttaagaattcatcggcggttggtcggcgcccaaccaccgcgctccactgcatccccggtcccaatgggcggtgccggctgtgccctcctcgtccatctctagctaatatatactcgaattagcctgataaaagattaaggagatggattaaaataagaaagccactattcgaaaggatgcctttagggcgagtatatatgcgcgtcttgttcgccggacttgacgcacaagctcactgcgaagcatagctaagcgagttctctttctaaaagtggttgattctagttctttcgatcgagcaaac

SEQ ID NO: 45 - DNA, 253 bp, Artificial Sequence
  Terminator
gatcgttcaaacatttggcaataaagtttcttaagattgaatcctgttgccggtcttgcgatgattatcatataatttctgttgaattacgttaagcatgtaataattaacatgtaatgcatgacgttatttatgagatgggtttttatgattagagtcccgcaattatacatttaatacgcgatagaaaacaaaatatagcgcgcaaactaggataaattatcgcgcgcggtgtcatctatgttactagatc

SEQ ID NO: 46 - protein, 607 aa, Populus balsamifera subsp. trichocarpa
MKRDHQETIGGGIGNRAESSSSSMETGKGKSWVEDDQDAGGMDELLAVLGYKIKSSDMADVAQKLEQLEMVLGSEDGISHLASDTVHYNPSDLSGWVQSMLSEFNNLPSTDLDSSILLSNNRDSLLGQPSTITPLDFPSNSQSKVFADDSEYDLRAIPGVAAYPQQELDKSNDRKRMKLTPIGSNIAPAPSVNSLQSPTASSTSSSSPQAMAVSGTLSEPTRPVVLVDSQETGVRLVHTLLACAEAIQQENLKLADALVKHIGLLAASQTGAMRKVATYFAEALARRIYKIFPQDYCLDSSCSDTLEMHFYETCPYLKFAHFTANQAILEAFANASRVHVIDFGLKQGMQWPALMQALALRPGGPPAFRLTGIGPPQPDNTDALQQVGWKLAQLAQTIGVEFEFRGFVANSLADLDAEMLGLLPPEVEAVAVNSVFELHRLLGRPGGIDKVLESIKAMRPKIVTIVEQEANHNGPVFLDRFTEALHYYSSLFDSLEGSGLTPPSQDLVMSELYLGRHICNVVACEGADRVERHETLAQWRTRFDSAGFDPVHLGSNAFKQASMLLALFAGGDGYRVEENNGCLMLGWHTRPLIATSAWQLAAGDSQQ

SEQ ID NO: 47 - protein, 600 aa, Populus balsamifera subsp. trichocarpa
MKREHPNLHPQQISDPSTLAAAGYSTSTSAMAPHNGKAKIWEEGEGHQADGGMDELLAVLGYKVRSSDMAEVAQKLEQLEEVMGHAQEDGLSHLASDSVHYNPSDLSTWLESMISELNPNLNFDPSADSLLAPAESSTITSIDFSDHKHHQQQKLFEESSSSDYDLKVIPGKAVFSQTQIDSRESKRLKTDLYQTSSSSSLSSATTLGSFGISTESTRPVVLVDSQENGIRLVHLLMACAEAVQESNFTLAEALVKQIGFLAVSQAGVMRKVATYFAEALARRIYKLCPQNSTDHSLSDILQIHFYETCPYLKFAHFTANQAILEAFEGKKRVHVIDFSMNQGMQWPALMQALAVRPGGPPAFRLTGIGPPAHDNTDHLQEVGWKLAQLAETIHVEFEYRGFVANSLADLDASMLELRPTESVAVNSVFELHKLLSRPGAIEKVLSVVKQMKPEIVTVVEQEANHNGPIFLDRFTESLHYYSTLFDSLEGSVSTQDKIMSEVYLGKQICNVVACEGPDRVERHETLTQWRTRLGSAGFAPVHLGSNAFKQASMLLALFAGGDGYRVEENNGCLMLGWHTRPLIATSAWRLNTNQPVVGAA

SEQ ID NO: 48 - protein, 602 aa, Populus balsamifera subsp. trichocarpa
MKREHSNLHPQQLTNPSSLAAGGYSLTSTGTMTSNNGKAKTWEEEKGRQADGGMDELLAVLGYKVRSSDMAEVAQKLEQLEEVMGHAQEDGLSHLASDSVHYNPSDLSTWLESMLSELNPNHHFDLSADSLLAPAESSTVTSIDFTDRKHHQQPKLFEESSSSEYDLKVIPGKAVFSPTQIDSRESKRLKTDLYQTSSSPSSSSTTLGSLVASTESTRPVVLVDSQENGVRLVHLLMACAEAVQENNLNLAEALVKQIGFLAVSQAGAMRKVATYFAEALARRIYKLYPQNSTDHSLSDILQIHFYETCPYLKFAHFTANQAILEAFEGKKRVHVIDFSMNQGMQWPALMQALALRPGGPPAFRLTGIGPPAHDNTDQLQEVGWKLAQLAETIHVEFEYRGFVANSLADLDASMLELRPTEFESVAVNSIFEFHKLLAIPGAMKKVLSVVKQMKPEIVTVVEQEANHNGPVFLDRFTESLHYYSTLFDSLEGSVSTQDKVMSEVYLAKQICNVVACEGSSRVERHETLTQWRTRLSSAGFAPVHLGSNAFKQASMLLALFAGGDGYRVEENNGCLMLGWHTRPLIATSAWRVNNHHPVGGAA

SEQ ID NO: 49 - protein, 619 aa, Populus balsamifera subsp. trichocarpa
MKRDHQETIGGAGNSIGNKAESSSSSMATGKGKLWVEDDQDAGGMDELLAVLGYKIKSSEMADVAQKLEQLEMVLGSEDGISHLASDTVHYNPSDLSGWVQSMLSELNNLPSSDLDSSTLLSNNQDSNPSTMTSLDFPNNSQSKAFVDDSEYDLRAIPGVAAYPQQEFDKSNDRKRMKLTLVGSNTAPTLAVNSLQSSNSSCTPSSPQAIMAVSGTLSEPTRPVVLIDSQETGVRLVHTLLACAEAIQQENLKLADALVKHIGVLAASQAGAMRKVATYFAEALARRIYKIFPQDHCLDSSYSDTLEMHFYETCPYLKFAHFTANQAILEAFANASRVHVIDFGLKQGMQWPALMQALALRPGGPPAFRLTGIGPPQPDNTDALQQVGWKLAQLAQTIGVEFEFRGFVASSLADLEAEMLDLRPPEVEAVAVNSVFELHRLLDRPGGIDKVLGSIKAMRPKIVTIVEQEANHNGPVFLDRFTEALHYYSSLFDSLEGSGVTPTSQDLVMSELYLGRQICNVVACEGADRVERHETLAQWRTRFDSAGFDPVHLGSNAFKQASMLLALFAGGDGYRVEENNGCLMLGWHTRPLIATSAWQLAAGDSRLRVNSAEFELPSQ

SEQ ID NO: 50 - protein, 607 aa, Populus tremula x Populus tremuloides
MKRDHQETIGGGIGNRGESSSSSMETGKGKSWVEDDQDAGGMDELLAVLGYKIKSSDMADVAQKLEQLEMALGSEDGISHLASDTVHYNPSDLSGWVQSMLSEFNNLPSTDLDSSILLSNNRDSLLGQPSTITPLDFPSNSQSKVFADDSEYDLRAIPGVAAYPQQELDKSNDRKRMKLNPIGSNIATAPSVNSLQSPTASPASSSSPQAMAVSGTLSESTRPVVLVDSQETGVRLVHTLLGCAEAIQQENLKLADALVKQIGLLAASQTGAMRKVATYFAEALARRIYKIFPQDYCLDSSCSDTLEMHFYETCPYLKFAHFTANQAILEAFANASRVHVIDFGLKQGMQWPALIQALALRPGGPPAFRLTGIGPPQPDNTDALQQVGWKLAQLAETIGVEFKFRGFVANSLADLDAEMLGLLPPEVEAVAVNSVFELHRLLGRPGGIDKVLGSIKAMRPKIVTIVEQEANHNGPVFLDRFTEALHYYSTLFDSLEGSGLTPPSQDLAMSELYLGRHICNVVACEGADRVERHETLAQWRTRFDSAGFDPVHLGSNAFKQASMLLALFAGGDGYRVEENNGCLMLGWHTRPLIATSAWQLAAGDSQQ

SEQ ID NO: 51 - protein, 622 aa, Populus tremula x Populus tremuloides
MKRDHQETIGGAGNSIGNKAESSSSSMTTGKGKLWVEDDQDAGGMDELLAVLGYKIKSSEMADVAQKLEQLEMVLGSEDGISHLASDTVHYNPSDLSGWVQSMLSEFNNLPSTDLDSSTLLSNNQDSNPSTMTSLDFSNNSQSKAFVDDSEYDLRAIPGVAAYPQQEFDKSNDRKRMKLTLAGSNTAPAPALAVNSLQSSSSSCTPSSSPQAIMAVSGTLSEPTRPVVLIDSQETGVRLVHTLLACAEAIQQENLKLADALVKHIGVLAASQAGAMRKVATYFAEALARRIYKIFPQNHCLDSSYSDTLEMHFYETCPYLKFAHFTANQAILEAFANASRVHVIDFGLKQGMQWPALMQALALRPGGPPAFRLTGIGPPQPDNTDALQQVGWKLAQLARTIGVEFEFRGFVASSLADLEAEMLDLRPPEVEAVAVNSVFELHRLLDRPGGIDKVLGSIKAMRPKIVTIVEQEANHNGPVFLDRFTEALHYYSSLFDSLEGSGVTPTSQDLVMSELYLGRQICNVVACEGADRVERHETLAQWRTRFDSAGFDPVHLGSNAFKQASMLLALFAGGDGYRVEENNGCLMLGWHTRPLIATSAWRLAAGDSRLRVNSAEFELPSQ

SEQ ID NO: 52 - protein, 602 aa, Populus tremula x Populus tremuloides
MKREHPNLHHQQISDPASLAAAGYSASTSTSAMAPNNGKAKIWAEGEGHQADGGVDELLAVLGYKVRSSDMAEVAQKLEQLEEVMGHAQEDGLSHLASDSVHYNPSDLSTWLQSMISELNPNLNFDPSADSLLAPAESSTITSIDFSDHKYHQQQKLFEESSSSDYDLKVIPGKAVFSQTHIDSRESKRLKTDLYQTSSSSSLSSATTLGSFGISTESARPVVLVDSQENGIRLVHLLMACAEAVQDSNFTLAEALVKQIGFLAVSQAGVMRKVATYFAEALARRIYKLCPQNSTDHSLSEILQIHFYETCPYLKFAHFTANQAILEAFEGKKRVHVIDFSMNQGMQWPALMQALALRPGGPPAFRLTGIGPPAHDNTDHLQEVGWKLAQLAETIHVEFEYRGFVANSLADLDASMLELRPTESVAVNSVFELHKLLSRPGAIEKVLSVVKQMKPEIVTVVEQEANHNGPIFLDRFTESLHYYSTLFDSLEGSVSTQDKIMSEVYLGKQICNVVACEGPDRVERHETLTQWRTRLGSAGFAPVHLGSNAFKQASMLLALFAGGDGYRVEENNGCLMLGWHTRPLIATSAWRLNTNQPVVGAA

SEQ ID NO: 53 - protein, 566 aa, Populus tremula x Populus tremuloides
MKREHSNLHPQQLTNPSSLAAGGYSFTSTGTMTSNNGKATTWEEEKGRQADGGMDELLAVLGYKVRSSDMAEVAQKLEQLEEVMGHAQEDGLSHLASDSVHYNPSDLSTWLESMLSELNPNHHFDLSADSLLGPAESSTVTSIDFTDRKHHQQPKLFEESSSSEYDLKVIPGKAVFSPTQIDSRESKRLKTDLYQTSSSPSSSSTTLGSLVASTESTRPVVLVDSQENGVRLVHLLMACAEAVQGDNLNLAEALVKQIGFLAVSQAGAMRKVATYFAEALARRIYKLYPQNSIDHSLSDILQIHFYETCPYLKFAHFTANQAILEAFEGKKRVHVIDFSMNQGMQWPALMQALALRPGGPPAFRLTGIGPPAHDNTDQLQEVGWKLAQLAETIHVEFEYRGFVANSLADLDASMLELRPPQFESVAVNSIFEFHKLLAIPGDMKKVLSVVKQMKPEIVTVVEQEANHNGPVFLDRFTESLHYYSTLFDSLEGSASTQDKVMSEVYLAKQICNVVACEGHSRVERHETLTQWRTRLSSAGFAPVHLGSNAFKQASMLLALFAGGEGV

SEQ ID NO: 54 - protein, 632 aa, Populus tremuloides
MKRDHQETIGGGIGNRGESSSSSMETGKGKSWVEDDQDAGGMDELLAVLGYKIKSSDMADVAQKLEQLEMALGSEDGISHLASDTVHYNPSDLSGWVQSMLSEFNNLPSTDLDSSILLSNNRDSLLGQPSTITPLDFPSNSQSKVFADDSEYDLRAIPGVAAYPQQELDKSNDRKRMKLNPIGSNIAPAPSVNSLQSPTASPASSSSPQAMAVSGTLSEPTRPVVLVDSQETGVRLVHTLLGCAEAIQQENLKLADALVKQIGLLAASQTGAMRKVATYFAEALARRIYKIFPQDYCLDSSCSDTLEMHFYETCPYLKFAHFTANQAILEAFANASRVHVIDFGLKQGMQWPALMQALALRPGGPPAFRLTGIGPPQPDNTDALQQVGWKLAQLAETIGVEFKFRGFVANSLADLDAEMLGLLPPEVEAVAVNSVFELHRLLGRPGGIDKVLGSIKAMRPKIVTIVEQEANHNGPVFLDRFTEALHYYSTLFDSLEGSGLTPPSQDLAMSELYLGRHICNVVACEGADRVERHETLAQWRTRFDSAGFDPVHLGSNAFKQASMLLALFAGGDGYRVEENNGCLMLGWHTRPLIATSAWQLAAGNGGHMWRILLLPCHLRREKILTALSSSRR

SEQ ID NO: 55 - protein, 669 aa, Populus tremuloides
MKRDHQETIGGAGNSIGNKAESPSSSMTTGKGKLWVEDDQDAGGMDELLAVLGYKIKSSEMADVAQKLEQLEMVLGSEDGISHLASDTVHYNPSDLSGWVQSMLSEFNNLPSTDLDSSTLLSNNQDSNPSTMTSLDFSNNSQSKAFVDDSEYDLRAIPGVAAYPQQEFDKSNDRKRMKLTLVGSNTAPAPALAVNSLQSSRSSCTPSSSPQAIMTVSGTLSEPTRPVVLIDSQETGVRLVHTLLACAEAIQQENLKLADALVKHIGVLAASQAGAMRKVATYFAEALARRIYKIFPQNHCLDSSYSDTLEMHFYETCPYLKFAHFTANQAILEAFANASRVHVIDFGLKQGMQWPALMQALALRPGGPPAFRLTGIGPPQPDNTDALQQVGWKLAQLARTIGVEFEFRGFVASSLADLEAEMLDLRPPEVEAVAVNSVFELHRLLDRPGGIDKVLGSIKAMRPKIVTIVEQEANHNGPVFLDRFTEALHYYSSLFDSLEGSGVTPTSQDLVMSELYLGRQICNVVACEGADRVERHETLAQWRTRFDSAGFDPVHLGSNAFKQASMLLALFAGGDGYRVEENSGCLMLGWHTRPLIATSAWRLAAGDSRLRVNSAEFELPNSQMDQESFFYLLLSGCPRFLSACIFFGLAFDISSLETLASFSFVTTSA

SEQ ID NO: 56 - protein, 636 aa, Populus tremuloides
MKREHSNLHPQQLTNPSSLAAGGYSFTSTGTMTSNNGKATTWEEEKGRQADGGMDELLAVLGYKVKSSDMAEVAQKLEQLEEVMGHAQEDGLSHLASDSVHYNPSDLSTWLESMLSELNPNHHFDLSAESLLGPAESSTVTSIDFTDRKHHQQPKLFEESSSSEYDLKVIPGKAVFSPTQIDSRESKRLKTDLYQTSSSPSSSSTTLGSLVASTESTRPVVLVDSQENGVRLVHLLMACAEAVQGDNLSLAEALVKQIGFLAVSQAGAMRKVATYFAEALARRIYKLYPQNSIDHSLSDILQIHFYETCPYLKFAHFTANQAILEAFEGKKRVHVIDFSMNQGMQWPALMQALALRPGGPPAFRLTGIGPPAHDNTDQLQEVGWKLAQLAETIHVEFEYRGFVANSLADLDASMLELRPPQFESVAVNSIFEFHKLLAIPGDMKKVLSVVKQMKPEIVTVVEQEANHNGPVFLDRFTESLHYYSTLFDSLEGSASTQDKVMSEVYLAKQICNVVACEGPSRVERHETLTQWRTRLSSAGFAPVHLGSNAFKQASMLLALFAGGDGYRVEENNGCLMLGWHTRPLIATSAWRVNNHYPGISENPPFMSGKQTHTEMIKVPLLPTLLRMRFCCCSCCC

SEQ ID NO: 57 - protein, 571 aa, Populus tremuloides
MKREHPNLHPQQISDPASLAAAGYSASTSTSAMAPNNGKAKIWAEGEGHQADGGVDELLAVLGYKVRSSDMAEVAQKLEQLEEVMGHAQEDGLSHLASDSVHYNPSDLSTWLQSMISELNPNLNFDPSADSLLAPAESSTITSIDFSDHKHHQQQKLFEESSSSDYDLKVIPGKAVFSQTHIDSRESKRLKTDLYQTSSSSSLSSATTLGSFGISTESARPVVLVDSQENGIRLVHLLMACAEAVQDSNFTLAEALVKQIGFLAVSQAGVMRKIHFYETCPYLKFAHFTANQAILEAFEGKKRVHVIDFSMNQGMQWPALMQALALRPGGPPAFRLTGIGPPAHDNTDHLQEVGWKLAQLAETIHVEFEYRGFVANSLADLDASMLELRPTESVAVNSVFELHKLLSRPGAIEKVLSVVKQMKPEIVTVVEQEANHNGPIFLDRFTESLHYYSTLFDSLEGSVSTQDKIMSEVYLGKQICNVVACEGPDRVERHETLTQWRTRLGSAGFAPVHLGSNAFKQASMLLALFAGGDGYRVEENNGCLMLGWHTRPLIATSAWRLNTNQPVVGAA

SEQ ID NO: 58 - protein, 623 aa, Brachypodium distachyon
MKREYQDGGGSRGGGDMGSSKDKMMVAAPAEEEDMDELLAALGYKVRASDMADVAQKLEQLEMAMGMGGVGAGAAPDDSFVAHLATDTVHSNPSDLSSWVESMLSELNAPPPPLPPAPQAPRLSSNSSTVTGGGGSGGGYFDGLPPSVDSSSSTYALRPIPSPVVTPAEPSADPAREPKRMRTGGGSTSSSSSSSSSLGGGGTMSSVVEAAPPAAPASAAANAPALPVVVVDTQEAGIRLVHALLACAEAVQQENLSAAEALVKQIPLLAASQGGAMRKVAAYFGEALARRVFRFRPQPDSSLLDAAFADLLHAHFYESCPYLKFAHFTANQAILEAFAGCRRVHVVDFGIKQGMQWPALLQALALRPGGPPSFRLTGVGPPQPDETDALQQVGWKLAQFAHTIRVDFQYRGLVAATLADLEPFMLQPEGEEDPNEEPEVIAVNSVFEMHRLLSQPGALEKVLGTVRAVRPRIVTVVEQEANHNSGSFLDRFTESLHYYSTMFDSLEGAGSGQSEISPGAAAGATDQVMSEVYLGRQICNVVACEGPERTERHETLGQWRGRLGQAGFETVHLGSNAYKQASTLLALFAGGDGYKVEEKDGCLTLGWHTRPLIATSAWRMAAP

SEQ ID NO: 59 - protein, 621 aa, Panicum virgatum
MKREYQDAGGSGGDMGSSKDKMMAAAAGEQDEEVDELLAALGYKVRSSDMADVAQKLEQLEMAMGMGGVGGAATAVDDGFVSHLATDTVHYNPSDLSSWVESMLSELNAPPPPLPTAPPAPRLASTSSTVTGGAAAGGGYFDLPPAVDSSSSTYALKPIPSPVAASADPSTDSTREPKRMRTGGGSTSSSSSSSSSLDGGRTRSSVVEAAPPATQASAAANAPAVPVVVVDTQEAGIRLVHALLACAEAVQQENFTAAEALVKQIPMLASSQGGAMRKVAAYFGEALARRVYRFRPAPDSSLLDAAFADLLHAHFYESCPYLKFAHFTANQAILEAFAGCRRVHVVDFGIKQGMQWPALLQALALRPGGPPSFRLTGVGPPQPDETDALQQVGWKLAQFAHTIRVDFQYRGLVAATLADLEPFMLQPDGEDTDDEPEVIAVNSVFELHRLLAQPGALEKVLGTVRAVRPRIVTVVEQEANHNSVSFLDRFTESLHYYSTMFDSLEGAGSGQSADAAPAAAGGTDQVMSEVYLGRQICNVVACEGAERTERHETLGQWRNRLGGAGFEPVHLGSNAYKQASTLLALFAGGDGYRVEEKDGCLTLGWHTRPLIATSAWRVAAP

SEQ ID NO: 60 - protein, 603 aa, Panicum virgatum
MKREYQDAGGSGGDMGSSKDNMMAAAAGEQNEEVDELLAALGYKVRSSDMADVAQKLEQLEMAMGMGGVGGAGAAADDGFVSHLVTDTVHYNPSDLSSWVENMLSELNAPPPRSRRLRGSRYFDLPPAVDSSSSTYALKPIPSPVAASADPSTDSTREPKRMRTGGGSTSSSSSSSSSLDGGRTRSSAVEAAPPATQASAAANAPAVPVVVVDTQEAGIRLVHALLACAEAVQQENFTAAEALVKQIPMLASSQGGAMRKVAAYFGEALARRVYRFRPAPDSSLLDAAFADLLHAHFYESCPYLKFAHFTANQAILEAFAGCRRVHVVDFGIKQGMQWPALLQALALRPGGPPSFRLTGVGPPQPDETDALQQVGWKLAQFAHTIRVDFQYRGLVAATLADLEPFMLQPDGEDTDDEPEVIAVNSVFELHRLLAQPGALEKVLGTVRAVRPRIVTVVEQEANHNSGSFLDRFTESLHYYSTMFDSLEGAGAGQSADAAPAAAGGTDQVMSEVYLGRQICNVVACEGAERTERHETLGQWRNRLGRAGFEPVHLGSNAYKQASTLLALFAGGDGYRVEEKDGCLTLGWHTRPLIATSAWRLAAP

SEQ ID NO: 61 - DNA, 1566 bp, Artificial Sequence
  Green tissue promoter
gtgaggagggggtgaaacactaaatcaagcgagatgcaatgtcaaccgagcctttccttgaggaagaaagcaaggtgatggaggaggcaattgtcaactgagatgcaaagtcaactttaaccggaaatcatccactcgtccaattggctggcggaggtgggggccccgagccaggagcaaaccttacccaaattagcttgcgaggttgagaggatcccatccaattaggtgtcgaatgtcgattgttgttggctccacctcggagatcacaagccatcattgacatgatagattgatatatcttatttcttccaattttgtggtgatagatctcagcaacctttcaaatcactacactgtgcaaaggatgatgttatttgtgttatttatccggaatccaaaatcagtattaagttatttgaagaaacatatagttagacgagttgtgtcatcttgatagatttcatatgatgaaattgagatgtctcgtgaaattaaatgggtgactcttaatcatacattttatgtgatacatatatatattatgtgccttattgattagttttcttacggtttatattttcagaaccaaagatttacctaccatgaaatcggagcataaattatgaattcaaattcctttggctcatggtttttaggaaaaaaaaagatttaatgagaggaactttcgcattttcaccgtttgtttgtgtaagttaagtaaattttgattcaagagtcacactggaaatgatctaaaagtgacaccaaccttggttttttccatttgtgcgaatgaaaaattaaactatatattgatgttaaagaaaaattagacagggatgtcgcttaaccttatgaaatcatgaccaaaaaccttatgaagccggttttacctctatggtcatgtcaacgggagtttttgtagcatttagcacgtgtaacgatttctttttgtcgaaagtgcatttgaacttgacacaatgcatttttaataagttattgcacattatcaagagtagttagtgcattgaaaatcgagaagtttccgtaaccaaattctaagctattcgttagtaatatctcccaagatattcattaaaaacatctggtacttcgttttcctcaaacctcctaactcttgattatcaatcctggacataaatctcaacatccacttgaaatgcatcctctgttctttttcccctaacaagaagcaaacgatcctcaatttcaccaaagcggggccaaagaaccatcactcataatcaacaaggatatctcatctatcttccaaccaaattaaaccccaaacatctctaaagcagcatcgaaaagaaaacagtccggaagtctctagctcaaaaactgtaaccccgtacctaattccagttgtctctgattacatcaattctcatgtcttaacactccattcgcacctccacaataaatagatcggcccttcatctccccttaccatcaaatccaatcccaaaaacacttgctcagacaccatcaaatccttcgcaaagtctttttcttacaaaaaaacaaacgaaagcaaca

SEQ ID NO: 62 - DNA, 1720 bp, Artificial Sequence
  Green tissue promoter
ttttatcctgtgatgccacattaatcagaatatatttttttctaaatagttaatgtttgggttcggcaaggatattcaaaattaaataatgaataaaatatagaataaaaaaattttgttcttgactactcgtgggttcttgttcaatctaggccttgggtctaagttatgggttaaattggatattaacaaaacattaaaggatatgataaatatgaaaagttaacctgaatttacttgagtatttttttttgttttttttttaatttaatattttaattttaattttattatttatcattgggttgatcgagaattgattttttttatggttttatgattcgtgtcgtgaatttaacaagttaattcaatttgatttaatattttatcttctcattattttaaaaaataatagcatccaatatatcgatatttgaaaatgatggcatctaatcttaatcatattttgagtctatggttgttattatttttagaaaataagttagcaatactttaatattttttatatattaaaacaatttaatctatcccgcaaacacatcgcaagttaatgatctaattataactataataaaacttgatttgagcaaaattcaatctcaaatatacaatatatagcattaatattgagttgaaatcaattatccaccaaatctatattgttgtttcaaaatacatttttgagtaaaggttttttcccccttttggttcaatgccttttattcttccaaattaatttcaatattttgtatccggaggaacatatttgtttcaaaaggtgtcagaaaatcaaagcccattgaaaatatataaacatatatagatataaaaactcaaggattcattccaaaatataagaacaaactgattgaattaatttgttattttaagaacactgtctatatgtttatatagtggtaggtagtgtttttaaaatcatatactaacttattataaaaataaatcataaaaaaggaacctcaagcatccctttgtaagctcgtatgtaggaatactcggagatcaaatgtccgaatgtcaaatgttaaggcaagtgaaatatccctaactttttagcaagcaaattgttgagtagctaaaatgaattattttaatatttttaaatcattttaatatattaatattaaaaaaaattaaatattttttttaatacattttcaataacaaacactttaaaatataatctttgtcacactcttaaacagtaacagcagaaagcatatgtgagtgatatagctatagttgctgtttgacacggacaatctccatctaaattcatgaataataaagttttgcctacacacccacttgaaatctcctcctagttttcctgatttgccatgctaactacaagaacaagatgctagctagtatcttgttctgtctctcgctctctctctatctctccagttgatagttgatagttgatagttgatagctgatacactcccacctttcccagaaagatgattgaggaactagtcactgtgttcgtgtaactaatactgttcatggcacctaacttgatcctctcttcaccagaccactataaaaaccctatctgtcctcctcataatcatctcactacacccaacacttctgcaagcacaactccattcaagaacatcaagagtataggccgccactgcaacaaaacagcactcctagctacttcaag

SEQ ID NO: 63 - DNA, 20 bp, Artificial Sequence
  Guide RNA
ggtcgtcgttgaagatgacc

SEQ ID NO: 64 - DNA, 20 bp, Artificial Sequence
  Guide RNA
ggtccaccaggacgaccggc

SEQ ID NO: 65 - DNA, 20 bp, Artificial Sequence
  Guide RNA
gatcatcgagacgcttgcag

SEQ ID NO: 66 - DNA, 20 bp, Artificial Sequence
  Guide RNA
tcctccacccactcaatgcc

SEQ ID NO: 67 - DNA, 20 bp, Artificial Sequence
  Guide RNA
ccaccacctctatccccaga

SEQ ID NO: 68 - DNA, 20 bp, Artificial Sequence
  Guide RNA
tccaagatgtgggacgaaga

SEQ ID NO: 69 - DNA, 20 bp, Artificial Sequence
  Guide RNA
gcagcagcagcaattgacgg

SEQ ID NO: 70 - DNA, 20 bp, Artificial Sequence
  Guide RNA
gcagcagcagcagcaattga

SEQ ID NO: 71 - DNA, 20 bp, Artificial Sequence
  Guide RNA
agtcgtcgttgaagatgacc

SEQ ID NO: 72 - DNA, 20 bp, Artificial Sequence
  Guide RNA
tgtccaccaggacgaccggc

SEQ ID NO: 73 - DNA, 426 bp, Artificial Sequence
  CaMV 35S promoter
caacatggtggagcacgacactctcgtctactccaagaatatcaaagatacagtctcagaagaccaaagggctattgagacttttcaacaaagggtaatatcgggaaacctcctcggattccattgcccagctatctgtcacttcatcaaaaggacagtagaaaaggaaggtggcacctacaaatgccatcattgcgataaaggaaaggctatcgttcaagatgcctctgccgacagtggtcccaaagatggacccccacccacgaggagcatcgtggaaaaagaagacgttccaaccacgtcttcaaagcaagtggattgatgtgatatctccactgacgtaagggatgacgcacaatcccactatccttcgcaagacccttcctctatataaggaagttcatttcatttggagaggacacgctg

SEQ ID NO: 74 - DNA, 835 bp, Artificial Sequence
  CaMV 35S promoter
agattagccttttcaatttcagaaagaatgctaacccacagatggttagagaggcttacgcagcaggtctcatcaagacgatctacccgagcaataatctccaggaaatcaaataccttcccaagaaggttaaagatgcagtcaaaagattcaggactaactgcatcaagaacacagagaaagatatatttctcaagatcagaagtactattccagtatggacgattcaaggcttgcttcacaaaccaaggcaagtaatagagattggagtctctaaaaaggtagttcccactgaatcaaaggccatggagtcaaagattcaaatagaggacctaacagaactcgccgtaaagactggcgaacagttcatacagagtctcttacgactcaatgacaagaagaaaatcttcgtcaacatggtggagcacgacacacttgtctactccaaaaatatcaaagatacagtctcagaagaccaaagggcaattgagacttttcaacaaagggtaatatccggaaacctcctcggattccattgcccagctatctgtcactttattgtgaagatagtggaaaaggaaggtggctcctacaaatgccatcattgcgataaaggaaaggccatcgttgaagatgcctctgccgacagtggtcccaaagatggacccccacccacgaggagcatcgtggaaaaagaagacgttccaaccacgtcttcaaagcaagtggattgatgtgatatctccactgacgtaagggatgacgcacaatcccactatccttcgcaagacccttcctctatataaggaagttcatttcatttggagagaacacg

SEQ ID NO: 75 - DNA, 442 bp, Arabidopsis thaliana
cgttgaacaacggaaactcgacttgccttccgcacaatacatcatttcttcttagctttttttcttcttcttcgttcatacagtttttttttgtttatcagcttacattttcttgaaccgtagctttcgttttcttctttttaactttccattcggagtttttgtatcttgtttcatagtttgtcccaggattagaatgattaggcatcgaaccttcaagaatttgattgaataaaacatcttcattcttaagatatgaagataatcttcaaaaggcccctgggaatctgaaagaagagaagcaggcccatttatatgggaaagaacaatagtatttcttatataggcccatttaagttgaaaacaatcttcaaaagtcccacatcgcttagataagaaaacgaagctgagtttatatacagctagagtcgaagtagtgatt

SEQ ID NO: 76 - DNA, 72 bp, Arabidopsis thaliana
tgatcaaaagtcccacatcgatcaggtgatatatagcagcttagtttatataatgatagagtcgacatagcg

SEQ ID NO: 77 - DNA, 4116 bp, Streptococcus pyogenes
atggacaagaagtactccattgggctcgatatcggcacaaacagcgtcggctgggccgtcattacggacgagtacaaggtgccgagcaaaaaattcaaagttctgggcaataccgatcgccacagcataaagaagaacctcattggcgccctcctgttcgactccggggagacggccgaagccacgcggctcaaaagaacagcacggcgcagatatacccgcagaaagaatcggatctgctacctgcaggagatctttagtaatgagatggctaaggtggatgactctttcttccataggctggaggagtcctttttggtggaggaggataaaaagcacgagcgccacccaatctttggcaatatcgtggacgaggtggcgtaccatgaaaagtacccaaccatatatcatctgaggaagaagcttgtagacagtactgataaggctgacttgcggttgatctatctcgcgctggcgcatatgatcaaatttcggggacacttcctcatcgagggggacctgaacccagacaacagcgatgtcgacaaactctttatccaactggttcagacttacaatcagcttttcgaagagaacccgatcaacgcatccggagttgacgccaaagcaatcctgagcgctaggctgtccaaatcccggcggctcgaaaacctcatcgcacagctccctggggagaagaagaacggcctgtttggtaatcttatcgccctgtcactcgggctgacccccaactttaaatctaacttcgacctggccgaagatgccaagcttcaactgagcaaagacacctacgatgatgatctcgacaatctgctggcccagatcggcgaccagtacgcagacctttttttggcggcaaagaacctgtcagacgccattctgctgagtgatattctgcgagtgaacacggagatcaccaaagctccgctgagcgctagtatgatcaagcgctatgatgagcaccaccaagacttgactttgctgaaggcccttgtcagacagcaactgcctgagaagtacaaggaaattttcttcgatcagtctaaaaatggctacgccggatacattgacggcggagcaagccaggaggaattttacaaatttattaagcccatcttggaaaaaatggacggcaccgaggagctgctggtaaagcttaacagagaagatctgttgcgcaaacagcgcactttcgacaatggaagcatcccccaccagattcacctgggcgaactgcacgctatcctcaggcggcaagaggatttctacccctttttgaaagataacagggaaaagattgagaaaatcctcacatttcggataccctactatgtaggccccctcgcccggggaaattccagattcgcgtggatgactcgcaaatcagaagagactatcactccctggaacttcgaggaagtcgtggataagggggcctctgcccagtccttcatcgaaaggatgactaactttgataaaaatctgcctaacgaaaaggtgcttcctaaacactctctgctgtacgagtacttcacagtttataacgagctcaccaaggtcaaatacgtcacagaagggatgagaaagccagcattcctgtctggagagcagaagaaagctatcgtggacctcctcttcaagacgaaccggaaagttaccgtgaaacagctcaaagaagattatttcaaaaagattgaatgtttcgactctgttgaaatcagcggagtggaggatcgcttcaacgcatccctgggaacgtatcacgatctcctgaaaatcattaaagacaaggacttcctggacaatgaggagaacgaggacattcttgaggacattgtcctcacccttacgttgtttgaagatagggagatgattgaagaacgcttgaaaacttacgctcatctcttcgacgacaaagtcatgaaacagctcaagaggcgccgatatacaggatgggggcggctgtcaagaaaactgatcaatgggatccgagacaagcagagtggaaagacaatcctggattttcttaagtccgatggatttgccaaccggaacttcatgcagttgatccatgatgactctctcacctttaaggaggacatccagaaagcacaagtttctggccagggggacagtctccacgagcacatcgctaatcttgcaggtagcccagctatcaaaaagggaatactgcagaccgttaaggtcgtggatgaactcgtcaaagtaatgggaaggcataagcccgagaatatcgttatcgagatggcccgagagaaccaaactacccagaagggacagaagaacagtagggaaaggatgaagaggattgaagagggtataaaagaactggggtcccaaatccttaaggaacacccagttgaaaacacccagcttcagaatgagaagctctacctgtactacctgcagaacggcagggacatgtacgtggatcaggaactggacatcaatcggctctccgactacgacgtggatcatatcgtgccccagtcttttctcaaagatgattctattgataataaagtgttgacaagatccgataaaaatagagggaagagtgataacgtcccctcagaagaagttgtcaagaaaatgaaaaattattggcggcagctgctgaacgccaaactgatcacacaacggaagttcgataatctgactaaggctgaacgaggtggcctgtctgagttggataaagccggcttcatcaaaaggcagcttgttgagacacgccagatcaccaagcacgtggcccaaattctcgattcacgcatgaacaccaagtacgatgaaaatgacaaactgattcgagaggtgaaagttattactctgaagtctaagctggtttcagatttcagaaaggactttcagttttataaggtgagagagatcaacaattaccaccatgcgcatgatgcctacctgaatgcagtggtaggcactgcacttatcaaaaaatatcccaagcttgaatctgaatttgtttacggagactataaagtgtacgatgttaggaaaatgatcgcaaagtctgagcaggaaataggcaaggccaccgctaagtacttcttttacagcaatattatgaattttttcaagaccgagattacactggccaatggagagattcggaagcgaccacttatcgaaacaaacggagaaacaggagaaatcgtgtgggacaagggtagggatttcgcgacagtccggaaggtcctgtccatgccgcaggtgaacatcgttaaaaagaccgaagtacagaccggaggcttctccaaggaaagtatcctcccgaaaaggaacagcgacaagctgatcgcacgcaaaaaagattgggaccccaagaaatacggcggattcgattctcctacagtcgcttacagtgtactggttgtggccaaagtggagaaagggaagtctaaaaaactcaaaagcgtcaaggaactgctgggcatcacaatcatggagcgatcaagcttcgaaaaaaaccccatcgactttctcgaggcgaaaggatataaagaggtcaaaaaagacctcatcattaagcttcccaagtactctctctttgagcttgaaaacggccggaaacgaatgctcgctagtgcgggcgagctgcagaaaggtaacgagctggcactgccctctaaatacgttaatttcttgtatctggccagccactatgaaaagctcaaaggatctcccgaagataatgagcagaagcagctgttcgtggaacaacacaaacactaccttgatgagatcatcgagcaaataagcgaattctccaaaagagtgatcctcgccgacgctaacctcgataaggtgctttctgcttacaataagcacagggataagcccatcagggagcaggcagaaaacattatccacttgtttactctgaccaacttgggcgcgcctgcagccttcaagtacttcgacaccaccatagacagaaagcggtacacctctacaaaggaggtcctggacgccacactgattcatcagtcaattacggggctctatgaaacaagaatcgacctctctcagctcggtggagacagcagggctgac

SEQ ID NO: 78 - DNA, 24 bp, Artificial Sequence
  Nuclear localization signal
cccaagaagaagaggaaggtgtga

SEQ ID NO: 79 - DNA, 84 bp, Artificial Sequence
  sgRNA scaffold
gttttagagctagaaatagcaagttaaaataaggctagtccgttatcaacttgaaaaagtggcaccgagtcggtgctttttttt

SEQ ID NO: 80 - DNA, 40 bp, Artificial Sequence
  U6 terminator
gttttgcaaaattttccagatcgatttcttcttcctctgt

SEQ ID NO: 81 - DNA, 305 bp, Arabidopsis thaliana
agaaatctcaaaattccggcagaacaattttgaatctcgatccgtagaaacgagacggtcattgttttagttccaccacgattatatttgaaatttacgctgagtgtgagtgagacttgcataagaaaataaaatctttagttgggaaaaaattcaataatataaatgggcttgagaaggaagcgagggataggcctttttctaaaataggcccatttaagctattaacaatcttcaaaagtaccacatcgcttaggtaaagaaagcagctgagtttatatatggttagagacgaagtagtgatt

SEQ ID NO: 82 - DNA, 319 bp, Arabidopsis thaliana
aaatatcagagatctcttacagttagtttcgttcttaatccaaactactgcagcctgacagacaaatgaggatgcaaacaattttaaagtttatctaacgctagctgttttgtttcttctctctggtgcaccaacgacggcgttttctcaatcataaagaggcttgttttacttaaggccaataatgttgatggatcgaaagaagagggcttttaataaacgagcccgtttaagctgtaaacgatgtcaaaaacatcccacatcgttcagttgaaaatagaagctctgtttatatattggtagagtcgactaagagatt

SEQ ID NO: 83 - DNA, 324 bp, Arabidopsis thaliana
tttactttaaattttttcttatgcagcctgtgatggataactgaatcaaacaaatggcgtctgggtttaagaagatctgttttggctatgttggacgaaacaagtgaacttttaggatcaacttcagtttatatatggagcttatatcgagcaataagataagtgggctttttatgtaatttaatgggctatcgtccatagattcactaatacccatgcccagtacccatgtatgcgtttcatataagctcctaatttctcccacatcgctcaaatctaaacaaatcttgttgtatatataacactgagggagcaacattggtc

SEQ ID NO: 84 - DNA, 102 bp, Arabidopsis thaliana
cataagcttatgatttcttttttcttacgaattttgcgtcccacatcggtaagcgagtgaagaaataactgctttatatatggctacaaagcaccattggtc

SEQ ID NO: 85 - DNA, 373 bp, Eucalyptus grandis
tctccgctggctaatttgattaaaatgaaaaggcccatcaaagaatttctcttgtcgaagagtaagcttgggtaggcggaccacctacccacccacccacccacccatggtgacccaattcaggtgtcgcgaactgcaataaaaagctttgctttgggaatcccgactcgttcgccaattgattaccgccccacagtttcgggtagggggaaaaaactcgtacaaggcccgcgccaaggaaaggtacgaggcccatgggctgggttcgactatttagtcttgcacggatctggcggaagaaaaaaaagtcccacatcggaccgcaactgacaaattgaacagtttttaagcggggaggagagaattactgggc